European Patent Application EP 4 295 673 A2, published December 27, 2023. Title: Introgression of two yield QTLs in Cucumis sativus plants. Applicant: Nunhems B.V. The sequence listing filed with the application follows.

SEQUENCE LISTING (40 sequences)

SEQ ID NO: 1 - DNA, 150 bp, Cucumis sativus
  source 1..150: mol_type = genomic DNA
ttgtataagaaagaagatcatacaaattatgaacatggttgataaattttggatgttgtacctaaaacatggaacagaatctcctatttaatccatcacaacaacaataatataaatagtaaataaacaaattaaataattttwcgaaag

SEQ ID NO: 2 - DNA, 150 bp, Cucumis sativus
  source 1..150: mol_type = genomic DNA
tgcttcttcttgaccatctttaccctctttcttgaccatgctgttgtacaggtccatctgtaaatggagacaatggcaagaaaaaagtaccgaccaattagtcatgtactagggttttccagctcaaaatacatttgggtcctgaagatc

SEQ ID NO: 3 - DNA, 150 bp, Cucumis sativus
  source 1..150: mol_type = genomic DNA
atttccttcttaacttctaaaaaagaggtagtaacttcagataacttttgggcatgatgagaactgtttaaagcggttagtgttggtaataacgaagattgcctcaataattctttccattgaggattcccatgggattttgttgatgat

SEQ ID NO: 4 - DNA, 150 bp, Cucumis sativus
  source 1..150: mol_type = genomic DNA
cagcacttcttctttccaatgtttcgatatctacaaacttttttgggatgtttttgtgggcttgttttcttttatgttttctcaattggagttgttgctttcaatttttttttacaaaaaggaaatccagaaatggcccccatatttaca

SEQ ID NO: 5 - DNA, 150 bp, Cucumis sativus
  source 1..150: mol_type = genomic DNA
gaaataaggcaaaagaataattcctccgaatgtcaatgtggatcaagactaagagtaagaaaattaaattaaactattaccatgattccagctgccacttactgctgtcagccgttgccctcatcctttactctgtggtccacaccttca

SEQ ID NO: 6 - DNA, 150 bp, Cucumis sativus
  source 1..150: mol_type = genomic DNA
caatttaacgaatattttattcagtcacaatatcatcttgatttcgaacatagcaaaatgaatcaaaatatttacgaccatagcaaaatctcaatgtctattagtgatagacactgagacaccaatagacactgataaatatctaaaact

SEQ ID NO: 7 - DNA, 150 bp, Cucumis sativus
  source 1..150: mol_type = genomic DNA
atattttactttagyattaagwcgttataacaattaagctaaaagaaggtaatgctaacgatactaattacttacagcttgagactcacacacagagactaaattaatctaggggagagtgaaatgatttaacttgtatgtagatgaagg

SEQ ID NO: 8 - DNA, 150 bp, Cucumis sativus
  source 1..150: mol_type = genomic DNA
gttgaggacttggtctatgtttgtcaagaataacacatttgatttcttcttttgatcagtttctaattgggatgaaaataccacactacactctttgatgctcacttttaggtcttgtggaagaagaattggactcttttggtggaagct

SEQ ID NO: 9 - DNA, 150 bp, Cucumis sativus
  source 1..150: mol_type = genomic DNA
ttaatttcttcttcttttagwattcttggaagttttttaagtattccattccttttgctaaatcagttatttttttacacaaaaaagaataacggcagcagactagaatccacattgataacatagattccatattaaaaattatgatga

SEQ ID NO: 10 - DNA, 150 bp, Cucumis sativus
  source 1..150: mol_type = genomic DNA
aaatgttgcataagaggagtacactttaattaaaattggaacagtcaatttttatgattttcagtttcagatattgagaacatttgaatgtaaatggggtgactcatctattgcgcaacccagacagcatccatatgctcctttcacaac

SEQ ID NO: 11 - DNA, 150 bp, Cucumis sativus
  source 1..150: mol_type = genomic DNA
tagaagatacgcaccccaactggcaacctaagggaacagccaacagaagaataataaacaaatgcatgaacctaggagaatttgaagtgcatcacaggaaattaagaaaaaagcaagcataaagcataactagaatagcataccccgcaa

SEQ ID NO: 12 - DNA, 150 bp, Cucumis sativus
  source 1..150: mol_type = genomic DNA
gtagtgtaaaagaaaaaaatatgaatgattgtagacatggcccacgttaatgaactttcagctatttttagtttgactttttgaactctactttgagtgcacttctgatcattaactagaaatattttggtaggtgcaagagctgacttg

SEQ ID NO: 13 - DNA, 150 bp, Cucumis sativus
  source 1..150: mol_type = genomic DNA
cataactctttattttgggtgatctattgtgatagacttgatgtataacttataaagttttcatagttcagttgcgtggtttattgcgatagacttgctgaagcatccaatgtgtgaaagtgaaggtgtgarttaccttctatkagakag

SEQ ID NO: 14 - DNA, 150 bp, Cucumis sativus
  source 1..150: mol_type = genomic DNA
ttattacaatggtcaaagtggcatttgttaattcatttaagaggaggagaaaaaacagatcttcagtcaaaaagagaagttgaatagtgaggcctaccgtgtgaaaaggcacgttatcctttcccataaattgaaaaagctctacatttt

SEQ ID NO: 15 - DNA, 150 bp, Cucumis sativus
  source 1..150: mol_type = genomic DNA
ctttgagcctctaatygaggttaaacaaatttcaatctttcataattgacttccgaagataatcaagagcaatccttgatagcaccaaaaatgtgttttctatctctacgtaattcgagctccttccttcattttactttcttatttggt

SEQ ID NO: 16 - DNA, 150 bp, Cucumis sativus
  source 1..150: mol_type = genomic DNA
atcttgtcagtctccggatttcatctagaatggttgttgaaggcagtctcagaattattaagagggccaaaggaaaagttttttaaaagctggatgaagtggatagaggtagattgaaagtttaaaattttaaaacaaagattggctggg

SEQ ID NO: 17 - DNA, 150 bp, Cucumis sativus
  source 1..150: mol_type = genomic DNA
tgaaactgagacgatatggagatttcagatttgacgcttcccaatgaatctagttggcttccttgggattaccatttcacattgttttttttttgtgtgtgtgtggtggggggactttggttttcttttcccttctaatttttttgctaa

SEQ ID NO: 18 - DNA, 150 bp, Cucumis sativus
  source 1..150: mol_type = genomic DNA
gtgttggagtaacacgaactgcagaatacaagaacagattattaggaaaaaaacctcataaatcatattcttacgaataagtaatttgggatatagtaagaaaaagaaaaaaaaaagatagaattatatgtatatagtacccatataatc

SEQ ID NO: 19 - DNA, 150 bp, Cucumis sativus
  source 1..150: mol_type = genomic DNA
cccagttcagatggaagttgcccattaaacttattgttgttcagaattagatattccaacctgatacaatcgccaatctctttcggtataattccggtgagttcattgaaggaaacattgagataagtcaggtggatcaacttaccaatg

SEQ ID NO: 20 - DNA, 150 bp, Cucumis sativus
  source 1..150: mol_type = genomic DNA
attggttgccactgacttgaatgttggaacaaattttcagtcatgaggagaatcagattatcatttggaaatgtgtatatatgcaataattaagtgaaaattttctattcgtgctcttttaacgaggaacaaatcttttttccattggta

SEQ ID NO: 21 - DNA, 150 bp, Cucumis sativus
  source 1..150: mol_type = genomic DNA
ctaaataccttatcttcatctactagtatatattttatcctgtttctcatactgagttgcatatttgagaagagggactatatgtgcttgtttctgtgtgtttatttataattctcatcttttggttgtcaatatgaagaatgctgattt

SEQ ID NO: 22 - DNA, 150 bp, Cucumis sativus
  source 1..150: mol_type = genomic DNA
ttataagatcaattactcaaartttcaaaaagccatctaatcaatgttagcctaaacgttttaagtcagataatgaacttaatatcatgatatgatatatatgaaagtgaaatctatttagaatctctataagacccactgtatccatca

SEQ ID NO: 23 - DNA, 150 bp, Cucumis sativus
  source 1..150: mol_type = genomic DNA
ggaattaaaagtgtatgaagaagagagacctccaattgagtagagcagttaatgagaggcctggctttgtgttttccatcaattaacttggaaagaaacaatgtgatatcagttggaaaatgatcagtttgatccaccaaccatctataw

SEQ ID NO: 24 - DNA, 150 bp, Cucumis sativus
  source 1..150: mol_type = genomic DNA
tagttcaaattacttcatgtttagattaatgtttaaagaaatggggagtctgccattaccagtaatcactctatgattgcaagtttagaatccaatgacaaagaaatgaaaaaatatttgtaagaacagttgtggaaaattacaactttt

SEQ ID NO: 25 - DNA, 150 bp, Cucumis sativus
  source 1..150: mol_type = genomic DNA
gatttggaggagattttccagcaacattccaagtagctacaaagattctattcatttaaacagaaagaagagaggcaaagaaggaattaaagacatagtccaaagaattcattgcctggaaacaacaaaatagagcatacataccggtaa

SEQ ID NO: 26 - DNA, 150 bp, Cucumis sativus
  source 1..150: mol_type = genomic DNA
cgtgtactttcttttcagtttaaccttaaaagtaatatttaactagtagtttggatttaaagttcgtgctttttcatttcaacaattagtcaactgtaataagatatcgttgcaactttattctattctatcatgtcacttgctgtgatc

SEQ ID NO: 27 - DNA, 150 bp, Cucumis sativus
  source 1..150: mol_type = genomic DNA
tgatkttgatctcttcccttaatcacgtaataggcaacttttgctttttctctttttgtgtgtgctttctgttcgacttaaaatatatatgagtgtgactaattatacttttaactacctaatatatatttatttccatccgattaagtt

SEQ ID NO: 28 - DNA, 150 bp, Cucumis sativus
  source 1..150: mol_type = genomic DNA
aaacgaaatgtttaaagaatgaaatattcccaattggtaaggagtaatcaatctacataataatgggtttgaactaaaaaaatgaaatttgtagctacaaaaaaattgaagctgagagagtaaattcaatggatgatcaaacaatttggg

SEQ ID NO: 29 - DNA, 150 bp, Cucumis sativus
  source 1..150: mol_type = genomic DNA
ttgtcagttaagaaatctccagtacaagaatttacaacaatacttgaacagccgcgatagatgatgtatgaaaacggattaaagatcgaaactaaaggaaggtggttccgacgatcatgagcccttgaatacagaagtcggagataatgg

SEQ ID NO: 30 - DNA, 150 bp, Cucumis sativus
  source 1..150: mol_type = genomic DNA
aawttttgttarattttagctcttaaactttttgaacttagtctctatactttcaaatttgtaataattttaactcaccataataaaccatatcagaattaagtgttattttttattgcctaacaacattttccatagtttataaacaaa

SEQ ID NO: 31 - DNA, 150 bp, Cucumis sativus
  source 1..150: mol_type = genomic DNA
ctgaaacctcttagccaactttctttggcaggcctttaaaaaccgggatcctgcttgtttgtcttacagttcagtgcttctatatcctaaggtaattgatattttcaaatcaagcggcttagtttggttcacagagctgttcaccgtcct

SEQ ID NO: 32 - DNA, 150 bp, Cucumis sativus
  source 1..150: mol_type = genomic DNA
aaaaccagtgagaaattgagaagcttgttgagtttactaaccggtgttttaatctcttgacaggtgaatgattacgtgcagtcgcacatacaaataaatgagtatcgggatcgtgttattctggtgagttactgaattctgggattcgac

SEQ ID NO: 33 - DNA, 150 bp, Cucumis sativus
  source 1..150: mol_type = genomic DNA
tatawatttgwatsttcaatttwaaattaaagaataaggtattccaataaagaaccaataggtctaataagctcgagaatcaaaagtaggaagactagtcaacaagagggacaactaactcaactccataaaaagtgttcagttatacaa

SEQ ID NO: 34 - DNA, 150 bp, Cucumis sativus
  source 1..150: mol_type = genomic DNA
ttcatggtttcaaccaccgtttctcaaacagacatcataacccattcatgttcaaacaccggcaactacaccactaacagcgtttacaagcaaaatctcgacaacctcctttcctccatcgcctccaacaccgaaattgattacggcttt

SEQ ID NO: 35 - DNA, 150 bp, Cucumis sativus
  source 1..150: mol_type = genomic DNA
agatatggtataaaagtgtygctacaactcactgttttcaaaactatatattaaaaattgtagacagagaaaatggagaaaagtaaaaacagctcttacattaccaatcaattgatccaaaaaatttaacttastaggcttgttcttytt

SEQ ID NO: 36 - DNA, 150 bp, Cucumis sativus
  source 1..150: mol_type = genomic DNA
tgtgggtaacggaagaagatgaatgcttggttggtattatcaccttcacgtcgatgttgaaggttttccacgagagtttgaaatcaatgtgttgaaagaacacatcagcaagagcttcgccctgatcttaagctgaagctatataatgam

SEQ ID NO: 37 - DNA, 150 bp, Cucumis sativus
  source 1..150: mol_type = genomic DNA
tgcaaacatttagaaccctggctgtttgtgtatctcaagaaatgaggaatttgtaaatgcagtaatcttaccatatgagaaagtgatagagcgagataaatcaacttgagcgtaactcaaatgttaagatattataatctcagtcaaaag

SEQ ID NO: 38 - DNA, 150 bp, Cucumis sativus
  source 1..150: mol_type = genomic DNA
aataatttggttcccaatttcactccgcatttaaactttgcttcttatgcctacaaattcttccccatcgtctgagttttacttttttaaccaaactccatctattttttcattcacttcattggtggattgaaacgcttctacgtttaa

SEQ ID NO: 39 - DNA, 150 bp, Cucumis sativus
  source 1..150: mol_type = genomic DNA
tattcaaactaaaactcccatttttcgattccttttaatattagttttcatatttctatggtctctgtttctttataaacctcacacactctagaatgttcactactttattaatatggttcttgggaattatggattcaataaactatt

SEQ ID NO: 40 - DNA, 150 bp, Cucumis sativus
  source 1..150: mol_type = genomic DNA
aatgcaagaaaagtagatccaagaagtgcgctttcaaggttgatagattctatttatgtatgaaaagatcatcttatctgcaattataatttacaatttggtatgcatatgcaagcatgaaataacattcatcaatacataaaagatatg